European Patent Specification EP 3 970 735 B1, published March 12, 2025. Title: USE OF COMPOSITION COMPRISING CHP (CYCLO-HIS PRO) AND PTH FOR PREVENTING, IMPROVING OR TREATING OF BONE LOSS RELATED DISEASE. Applicant: NovMetaPharma Co., Ltd. The sequence listing filed with the application follows.

SEQUENCE LISTING (18 sequences)

SEQ ID NO: 1 - protein, 84 aa, Artificial
  PTH
SVSEIQLMHNLGKHLNSMERVEWLRKKLQDVHNFVALGAPLAPRDAGSQRPRKKEDNVLVESHEKSLGEADKANVDVLTKAKSQ

SEQ ID NO: 2 - protein, 34 aa, Artificial
  PTH1-34
SVSEIQLMHNLGKHLNSMERVEWLRKKLQDVHNF

SEQ ID NO: 3 - DNA, 20 bp, Artificial
  ALP forward primer
agatggcctggatctcatca

SEQ ID NO: 4 - DNA, 20 bp, Artificial
  ALP reverse primer
cagtgcggttccagacatag

SEQ ID NO: 5 - DNA, 20 bp, Artificial
  BMP2 forward primer
tggaagtggcccatttagag

SEQ ID NO: 6 - DNA, 20 bp, Artificial
  BMP2 reverse primer
tgacgcttttctcgtttgtg

SEQ ID NO: 7 - DNA, 18 bp, Artificial
  Osteocalcin forward primer
ctgctcactctgctgacc

SEQ ID NO: 8 - DNA, 18 bp, Artificial
  Osteocalcin reverse primer
ttgtcagactcagggccg

SEQ ID NO: 9 - DNA, 20 bp, Artificial
  Osterix forward primer
gaagtccaatggggatctga

SEQ ID NO: 10 - DNA, 20 bp, Artificial
  Osterix reverse primer
agaatccctttccctctcca

SEQ ID NO: 11 - DNA, 21 bp, Artificial
  Runx2 forward primer
aagtgcggtgcaaactttctc

SEQ ID NO: 12 - DNA, 22 bp, Artificial
  Runx2 reverse primer
tgcttgcagccttaaatattcc

SEQ ID NO: 13 - DNA, 19 bp, Artificial
  Col1a1 forward primer
ctaacgtggttcgtgaccg

SEQ ID NO: 14 - DNA, 20 bp, Artificial
  Col1a1 reverse primer
gctgcggatgttctcaatct

SEQ ID NO: 15 - DNA, 21 bp, Artificial
  OPG forward primer
ggaatagatgtcaccctgtgt

SEQ ID NO: 16 - DNA, 23 bp, Artificial
  OPG reverse primer
aaaacactcagccaatttggtat

SEQ ID NO: 17 - DNA, 18 bp, Artificial
  Beta-actin forward primer
gggaaggtgacagcattg

SEQ ID NO: 18 - DNA, 23 bp, Artificial
  Beta-actin reverse primer
atgaagtattaaggcggaagatt